European Patent Specification EP 3 740 074 B1, published November 6, 2024. Title: PIC1 INHIBITION OF MYELOPEROXIDASE OXIDATIVE ACTIVITY IN AN ANIMAL MODEL. Applicant: REALTA HOLDINGS, LLC. The sequence listing filed with the application follows.

SEQUENCE LISTING (45 sequences)

SEQ ID NO: 1 - protein, 15 aa, Artificial Sequence
  Description of Artificial Sequence: Synthetic peptide
IALILEPICCQERAA

SEQ ID NO: 2 - protein, 15 aa, Artificial Sequence
  Description of Artificial Sequence: Synthetic peptide
  MOD_RES (1)..(1): Sarcosine
XALILEPICCQERAA

SEQ ID NO: 3 - protein, 15 aa, Artificial Sequence
  Description of Artificial Sequence: Synthetic peptide
  MOD_RES (2)..(2): Sarcosine
IXLILEPICCQERAA

SEQ ID NO: 4 - protein, 15 aa, Artificial Sequence
  Description of Artificial Sequence: Synthetic peptide
  MOD_RES (3)..(3): Sarcosine
IAXILEPICCQERAA

SEQ ID NO: 5 - protein, 15 aa, Artificial Sequence
  Description of Artificial Sequence: Synthetic peptide
  MOD_RES (4)..(4): Sarcosine
IALXLEPICCQERAA

SEQ ID NO: 6 - protein, 15 aa, Artificial Sequence
  Description of Artificial Sequence: Synthetic peptide
  MOD_RES (5)..(5): Sarcosine
IALIXEPICCQERAA

SEQ ID NO: 7 - protein, 15 aa, Artificial Sequence
  Description of Artificial Sequence: Synthetic peptide
  MOD_RES (6)..(6): Sarcosine
IALILXPICCQERAA

SEQ ID NO: 8 - protein, 15 aa, Artificial Sequence
  Description of Artificial Sequence: Synthetic peptide
  MOD_RES (7)..(7): Sarcosine
IALILEXICCQERAA

SEQ ID NO: 9 - protein, 15 aa, Artificial Sequence
  Description of Artificial Sequence: Synthetic peptide
  MOD_RES (8)..(8): Sarcosine
IALILEPXCCQERAA

SEQ ID NO: 10 - protein, 15 aa, Artificial Sequence
  Description of Artificial Sequence: Synthetic peptide
  MOD_RES (9)..(9): Sarcosine
IALILEPIXCQERAA

SEQ ID NO: 11 - protein, 15 aa, Artificial Sequence
  Description of Artificial Sequence: Synthetic peptide
  MOD_RES (10)..(10): Sarcosine
IALILEPICXQERAA

SEQ ID NO: 12 - protein, 14 aa, Artificial Sequence
  Description of Artificial Sequence: Synthetic peptide
  MOD_RES (10)..(10): Sarcosine
ALILEPICCXERAA

SEQ ID NO: 13 - protein, 15 aa, Artificial Sequence
  Description of Artificial Sequence: Synthetic peptide
  MOD_RES (12)..(12): Sarcosine
IALILEPICCQXRAA

SEQ ID NO: 14 - protein, 15 aa, Artificial Sequence
  Description of Artificial Sequence: Synthetic peptide
  MOD_RES (13)..(13): Sarcosine
IALILEPICCQEXAA

SEQ ID NO: 15 - protein, 15 aa, Artificial Sequence
  Description of Artificial Sequence: Synthetic peptide
  MOD_RES (14)..(14): Sarcosine
IALILEPICCQERXA

SEQ ID NO: 16 - protein, 15 aa, Artificial Sequence
  Description of Artificial Sequence: Synthetic peptide
  MOD_RES (15)..(15): Sarcosine
IALILEPICCQERAX

SEQ ID NO: 17 - protein, 15 aa, Artificial Sequence
  Description of Artificial Sequence: Synthetic peptide
  MOD_RES (1)..(1): N-term dPEG24
  MOD_RES (15)..(15): C-term dPEG24
IALILEPICCQERAA

SEQ ID NO: 18 - protein, 15 aa, Artificial Sequence
  Description of Artificial Sequence: Synthetic peptide
  MOD_RES (1)..(1): N-term dPEG24
IALILEPICCQERAA

SEQ ID NO: 19 - protein, 15 aa, Artificial Sequence
  Description of Artificial Sequence: Synthetic peptide
  MOD_RES (15)..(15): C-term dPEG24
IALILEPICCQERAA

SEQ ID NO: 20 - protein, 15 aa, Artificial Sequence
  Description of Artificial Sequence: Synthetic peptide
  MOD_RES (15)..(15): C-term dPEG20
IALILEPICCQERAA

SEQ ID NO: 21 - protein, 15 aa, Artificial Sequence
  Description of Artificial Sequence: Synthetic peptide
  MOD_RES (15)..(15): C-term dPEG16
IALILEPICCQERAA

SEQ ID NO: 22 - protein, 15 aa, Artificial Sequence
  Description of Artificial Sequence: Synthetic peptide
  MOD_RES (15)..(15): C-term dPEG12
IALILEPICCQERAA

SEQ ID NO: 23 - protein, 15 aa, Artificial Sequence
  Description of Artificial Sequence: Synthetic peptide
  MOD_RES (15)..(15): C-term dPEG08
IALILEPICCQERAA

SEQ ID NO: 24 - protein, 15 aa, Artificial Sequence
  Description of Artificial Sequence: Synthetic peptide
  MOD_RES (15)..(15): C-term dPEG06
IALILEPICCQERAA

SEQ ID NO: 25 - protein, 15 aa, Artificial Sequence
  Description of Artificial Sequence: Synthetic peptide
  MOD_RES (15)..(15): C-term dPEG04
IALILEPICCQERAA

SEQ ID NO: 26 - protein, 15 aa, Artificial Sequence
  Description of Artificial Sequence: Synthetic peptide
  MOD_RES (15)..(15): C-term dPEG03
IALILEPICCQERAA

SEQ ID NO: 27 - protein, 15 aa, Artificial Sequence
  Description of Artificial Sequence: Synthetic peptide
  MOD_RES (15)..(15): C-term dPEG02
IALILEPICCQERAA

SEQ ID NO: 28 - protein, 15 aa, Artificial Sequence
  Description of Artificial Sequence: Synthetic peptide
  MOD_RES (9)..(9): Sarcosine
IALILEPIXAQERAA

SEQ ID NO: 29 - protein, 14 aa, Artificial Sequence
  Description of Artificial Sequence: Synthetic peptide
  MOD_RES (9)..(9): Sarcosine
IALILEPIXQERAA

SEQ ID NO: 30 - protein, 15 aa, Artificial Sequence
  Description of Artificial Sequence: Synthetic peptide
  MOD_RES (7)..(7): Sarcosine
  MOD_RES (9)..(9): Sarcosine
IALILEXIXCQERAA

SEQ ID NO: 31 - protein, 15 aa, Artificial Sequence
  Description of Artificial Sequence: Synthetic peptide
  MOD_RES (15)..(15): C-term dPEG24
  MOD_RES (6)..(6): Sarcosine
IALILXPICCQERAA

SEQ ID NO: 32 - protein, 15 aa, Artificial Sequence
  Description of Artificial Sequence: Synthetic peptide
  MOD_RES (15)..(15): C-term dPEG24
  MOD_RES (11)..(11): Sarcosine
IALILEPICCXERAA

SEQ ID NO: 33 - protein, 15 aa, Artificial Sequence
  Description of Artificial Sequence: Synthetic peptide
  MOD_RES (15)..(15): C-term dPEG24
  MOD_RES (13)..(13): Sarcosine
IALILEPICCQEXAA

SEQ ID NO: 34 - protein, 15 aa, Artificial Sequence
  Description of Artificial Sequence: Synthetic peptide
  MOD_RES (15)..(15): C-term dPEG24
  MOD_RES (14)..(14): Sarcosine
IALILEPICCQERXA

SEQ ID NO: 35 - protein, 15 aa, Artificial Sequence
  Description of Artificial Sequence: Synthetic peptide
  MOD_RES (6)..(7): Sarcosine
IALILXXICCQERAA

SEQ ID NO: 36 - protein, 15 aa, Artificial Sequence
  Description of Artificial Sequence: Synthetic peptide
  MOD_RES (6)..(6): Sarcosine
  MOD_RES (9)..(9): Sarcosine
IALILXPIXCQERAA

SEQ ID NO: 37 - protein, 15 aa, Artificial Sequence
  Description of Artificial Sequence: Synthetic peptide
  MOD_RES (7)..(7): Sarcosine
  MOD_RES (11)..(11): Sarcosine
IALILEXICCXERAA

SEQ ID NO: 38 - protein, 15 aa, Artificial Sequence
  Description of Artificial Sequence: Synthetic peptide
  MOD_RES (9)..(9): Sarcosine
  MOD_RES (11)..(11): Sarcosine
IALILEPIXCXERAA

SEQ ID NO: 39 - protein, 15 aa, Artificial Sequence
  Description of Artificial Sequence: Synthetic peptide
  MOD_RES (7)..(7): Sarcosine
  MOD_RES (13)..(13): Sarcosine
IALILEXICCQEXAA

SEQ ID NO: 40 - protein, 15 aa, Artificial Sequence
  Description of Artificial Sequence: Synthetic peptide
  MOD_RES (9)..(9): Sarcosine
  MOD_RES (13)..(13): Sarcosine
IALILEPIXCQEXAA

SEQ ID NO: 41 - protein, 15 aa, Artificial Sequence
  Description of Artificial Sequence: Synthetic peptide
  MOD_RES (7)..(7): Sarcosine
  MOD_RES (14)..(14): Sarcosine
IALILEXICCQERXA

SEQ ID NO: 42 - protein, 15 aa, Artificial Sequence
  Description of Artificial Sequence: Synthetic peptide
  MOD_RES (9)..(9): Sarcosine
  MOD_RES (14)..(14): Sarcosine
IALILEPIXCQERXA

SEQ ID NO: 43 - protein, 15 aa, Artificial Sequence
  Description of Artificial Sequence: Synthetic peptide
  MOD_RES (15)..(15): C-term dPEG24
IALILAPICCQARAA

SEQ ID NO: 44 - protein, 15 aa, Artificial Sequence
  Description of Artificial Sequence: Synthetic peptide
  MOD_RES (9)..(9): Sarcosine
IALILAPIXCQARAA

SEQ ID NO: 45 - protein, 15 aa, Artificial Sequence
  Description of Artificial Sequence: Synthetic peptide
  MOD_RES (7)..(7): Sarcosine
IALILAXICCQARAA